European Patent Specification EP 4 380 968 B1, published October 1, 2025. Title: Pharmaceutical Compositions Comprising HLA Fusion Proteins. Applicant: ImmunOs Therapeutics AG. The sequence listing filed with the application follows.

SEQUENCE LISTING (21 sequences)

SEQ ID NO: 1 - protein, 280 aa, synthetic construct
  REGION 1..280: note = HLA-B57:01 extracellular domain A46E V97R
GSHSMRYFYTAMSRPGRGEPRFIAVGYVDDTQFVRFDSDAASPRMEPRAPWIEQEGPEYWDGETRNMKASAQTYRENLRIALRYYNQSEAGSHIIQRMYGCDVGPDGRLLRGHDQSAYDGKDYIALNEDLSSWTAADTAAQITQRKWEAARVAEQLRAYLEGLCVEWLRRYLENGKETLQRADPPKTHVTHHPISDHEATLRCWALGFYPAEITLTWQRDGEDQTQDTELVETRPAGDRTFQKWAAVVVPSGEEQRYTCHVQHEGLPKPLTLRWEPSSQS

SEQ ID NO: 2 - protein, 228 aa, synthetic construct
  REGION 1..228: note = Optimized IgG4 Fc
ESKYGPPCPPCPAPEFLGGPSVFLFPPKPKDTLMISRTPEVTCVVVDVSQEDPEVQFNWYVDGVEVHNAKTKPREEQFNSTYRVVSVLTVLHQDWLNGKEYKCKVSNKGLPSSIEKTISKAKGQPREPQVYTLPPSQEEMTKNQVSLTCLVKGFYPSDIAVEWESNGQPENNYKTTPPVLDSDGSFFLYSRLTVDKSRWQEGNVFSCSVMHEALHNHYTQKSLSLSLG

SEQ ID NO: 3 - protein, 10 aa, synthetic construct
  REGION 1..10: note = peptide linker
GGGGSGGGGS

SEQ ID NO: 4 - protein, 21 aa, synthetic construct
  REGION 1..21: note = HLA fusion protein secretory signal
AAAMNFGLRLIFLVLTLKGVQ

SEQ ID NO: 5 - protein, 518 aa, synthetic construct
  REGION 1..518: note = variant HLA-B57 extracellular domain IgG4 Fc fusion protein,lacking secretory signal
GSHSMRYFYTAMSRPGRGEPRFIAVGYVDDTQFVRFDSDAASPRMEPRAPWIEQEGPEYWDGETRNMKASAQTYRENLRIALRYYNQSEAGSHIIQRMYGCDVGPDGRLLRGHDQSAYDGKDYIALNEDLSSWTAADTAAQITQRKWEAARVAEQLRAYLEGLCVEWLRRYLENGKETLQRADPPKTHVTHHPISDHEATLRCWALGFYPAEITLTWQRDGEDQTQDTELVETRPAGDRTFQKWAAVVVPSGEEQRYTCHVQHEGLPKPLTLRWEPSSQSGGGGSGGGGSESKYGPPCPPCPAPEFLGGPSVFLFPPKPKDTLMISRTPEVTCVVVDVSQEDPEVQFNWYVDGVEVHNAKTKPREEQFNSTYRVVSVLTVLHQDWLNGKEYKCKVSNKGLPSSIEKTISKAKGQPREPQVYTLPPSQEEMTKNQVSLTCLVKGFYPSDIAVEWESNGQPENNYKTTPPVLDSDGSFFLYSRLTVDKSRWQEGNVFSCSVMHEALHNHYTQKSLSLSLG

SEQ ID NO: 6 - protein, 99 aa, Homo sapiens [sequence omitted]

SEQ ID NO: 7 - protein, 518 aa, synthetic construct
GSHSMRYFSTSVSRPGSGEPRFIAVGYVDDTQFVRFDSDAASQRMEPRAPWIEQERPEYWDQETRNVKAQSQTDRVDLGTLRGYYNQSEAGSHTIQIMYGCDVGSDGRFLRGYEQHAYDGKDYIALNEDLRSWTAADMAAQITQRKWEAARWAEQLRAYLEGTCVEWLRRYLENGKETLQRTDPPKTHMTHHPISDHEATLRCWALGFYPAEITLTWQRDGEDQTQDTELVETRPAGDGTFQKWAAVVVPSGEEQRYTCHVQHEGLPKPLTLRWELSSQPGGGGSGGGGSESKYGPPCPPCPAPEFLGGPSVFLFPPKPKDTLMISRTPEVTCVVVDVSQEDPEVQFNWYVDGVEVHNAKTKPREEQFNSTYRVVSVLTVLHQDWLNGKEYKCKVSNKGLPSSIEKTISKAKGQPREPQVYTLPPSQEEMTKNQVSLTCLVKGFYPSDIAVEWESNGQPENNYKTTPPVLDSDGSFFLYSRLTVDKSRWQEGNVFSCSVMHEALHNHYTQKSLSLSLG

SEQ ID NO: 8 - protein, 518 aa, synthetic construct
GSHSMRYFYTAMSRPGRGEPRFIAVGYVDDTQFVRFDSDAASPRMAPRAPWIEQEGPEYWDGETRNMKASAQTYRENLRIALRYYNQSEAGSHIIQVMYGCDVGPDGRLLRGHDQSAYDGKDYIALNEDLSSWTAADTAAQITQRKWEAARVAEQLRAYLEGLCVEWLRRYLENGKETLQRADPPKTHVTHHPISDHEATLRCWALGFYPAEITLTWQRDGEDQTQDTELVETRPAGDRTFQKWAAVVVPSGEEQRYTCHVQHEGLPKPLTLRWEPSSQSGGGGSGGGGSESKYGPPCPPCPAPEFLGGPSVFLFPPKPKDTLMISRTPEVTCVVVDVSQEDPEVQFNWYVDGVEVHNAKTKPREEQFNSTYRVVSVLTVLHQDWLNGKEYKCKVSNKGLPSSIEKTISKAKGQPREPQVYTLPPSQEEMTKNQVSLTCLVKGFYPSDIAVEWESNGQPENNYKTTPPVLDSDGSFFLYSRLTVDKSRWQEGNVFSCSVMHEALHNHYTQKSLSLSLG

SEQ ID NO: 9 - protein, 518 aa, synthetic construct
GSHSMRYFYTAMSRPGRGEPRFIAVGYVDDTQFVRFDSDAASPRTEPRAPWIEQEGPEYWDGETRNMKASAQTYRENLRIALRYYNQSEAGSHIIQRMYGCDLGPDGRLLRGHDQSAYDGKDYIALNEDLSSWTAADTAAQITQRKWEAARVAEQLRAYLEGLCVEWLRRYLENGKETLQRADPPKTHVTHHPVSDHEATLRCWALGFYPAEITLTWQRDGEDQTQDTELVETRPAGDRTFQKWAAVVVPSGEEQRYTCHVQHEGLPKPLTLRWEPSSQSGGGGSGGGGSESKYGPPCPPCPAPEFLGGPSVFLFPPKPKDTLMISRTPEVTCVVVDVSQEDPEVQFNWYVDGVEVHNAKTKPREEQFNSTYRVVSVLTVLHQDWLNGKEYKCKVSNKGLPSSIEKTISKAKGQPREPQVYTLPPSQEEMTKNQVSLTCLVKGFYPSDIAVEWESNGQPENNYKTTPPVLDSDGSFFLYSRLTVDKSRWQEGNVFSCSVMHEALHNHYTQKSLSLSLG

SEQ ID NO: 10 - protein, 518 aa, synthetic construct
CSHSMRYFYTAVSRPGRGEPRFIAVGYVDDTQFVQFDSDAASPRGEPRAPWVEQEGPEYWDRETQKYKRQAQTDRVSLRNLRGYYNQSEAGSHTLQRMYGCDLGPDGRLLRGYNQFAYDGKDYIALNEDLRSWTAADKAAQITQRKWEAAREAEQRRAYLEGTCVEWLRRYLENGKKTLQRAEHPKTHVTHHPVSDHEATLRCWALGFYPAEITLTWQRDGEDQTQDTELVETRPAGDGTFQKWAAVVVPSGEEQRYTCHVQHEGLPEPLTLRWGPSSQPGGGGSGGGGSESKYGPPCPPCPAPEFLGGPSVFLFPPKPKDTLMISRTPEVTCVVVDVSQEDPEVQFNWYVDGVEVHNAKTKPREEQFNSTYRVVSVLTVLHQDWLNGKEYKCKVSNKGLPSSIEKTISKAKGQPREPQVYTLPPSQEEMTKNQVSLTCLVKGFYPSDIAVEWESNGQPENNYKTTPPVLDSDGSFFLYSRLTVDKSRWQEGNVFSCSVMHEALHNHYTQKSLSLSLG

SEQ ID NO: 11 - protein, 518 aa, synthetic construct
GSHSMRYFSTSVSRPGSGEPRFIAVGYVDDTQFVRFDSDAASQRMAPRAPWIEQERPEYWDQETRNVKAQSQTDRVDLGTLRGYYNQSEAGSHTIQIMYGCDVGSDGRFLRGYEQHAYDGKDYIALNEDLRSWTAADMAAQITQRKWEAARWAEQLRAYLEGTCVEWLRRYLENGKETLQRTDPPKTHMTHHPISDHEATLRCWALGFYPAEITLTWQRDGEDQTQDTELVETRPAGDGTFQKWAAVVVPSGEEQRYTCHVQHEGLPKPLTLRWELSSQPGGGGSGGGGSESKYGPPCPPCPAPEFLGGPSVFLFPPKPKDTLMISRTPEVTCVVVDVSQEDPEVQFNWYVDGVEVHNAKTKPREEQFNSTYRVVSVLTVLHQDWLNGKEYKCKVSNKGLPSSIEKTISKAKGQPREPQVYTLPPSQEEMTKNQVSLTCLVKGFYPSDIAVEWESNGQPENNYKTTPPVLDSDGSFFLYSRLTVDKSRWQEGNVFSCSVMHEALHNHYTQKSLSLSLG

SEQ ID NO: 12 - protein, 518 aa, synthetic construct
GSHSMRYFSTSVSRPGSGEPRFIAVGYVDDTQFVRFDSDAASQRMEPRAPWIEQERPEYWDQETRNVKAQSQTDRVDLGTLRGYYNQSEAGSHTIQRMYGCDVGSDGRFLRGYEQHAYDGKDYIALNEDLRSWTAADMAAQITQRKWEAARWAEQLRAYLEGTCVEWLRRYLENGKETLQRTDPPKTHMTHHPISDHEATLRCWALGFYPAEITLTWQRDGEDQTQDTELVETRPAGDGTFQKWAAVVVPSGEEQRYTCHVQHEGLPKPLTLRWELSSQPGGGGSGGGGSESKYGPPCPPCPAPEFLGGPSVFLFPPKPKDTLMISRTPEVTCVVVDVSQEDPEVQFNWYVDGVEVHNAKTKPREEQFNSTYRVVSVLTVLHQDWLNGKEYKCKVSNKGLPSSIEKTISKAKGQPREPQVYTLPPSQEEMTKNQVSLTCLVKGFYPSDIAVEWESNGQPENNYKTTPPVLDSDGSFFLYSRLTVDKSRWQEGNVFSCSVMHEALHNHYTQKSLSLSLG

SEQ ID NO: 13 - protein, 518 aa, synthetic construct
GSHSMRYFSTSVSRPGSGEPRFIAVGYVDDTQFVRFDSDAASQRMAPRAPWIEQERPEYWDQETRNVKAQSQTDRVDLGTLRGYYNQSEAGSHTIQRMYGCDVGSDGRFLRGYEQHAYDGKDYIALNEDLRSWTAADMAAQITQRKWEAARWAEQLRAYLEGTCVEWLRRYLENGKETLQRTDPPKTHMTHHPISDHEATLRCWALGFYPAEITLTWQRDGEDQTQDTELVETRPAGDGTFQKWAAVVVPSGEEQRYTCHVQHEGLPKPLTLRWELSSQPGGGGSGGGGSESKYGPPCPPCPAPEFLGGPSVFLFPPKPKDTLMISRTPEVTCVVVDVSQEDPEVQFNWYVDGVEVHNAKTKPREEQFNSTYRVVSVLTVLHQDWLNGKEYKCKVSNKGLPSSIEKTISKAKGQPREPQVYTLPPSQEEMTKNQVSLTCLVKGFYPSDIAVEWESNGQPENNYKTTPPVLDSDGSFFLYSRLTVDKSRWQEGNVFSCSVMHEALHNHYTQKSLSLSLG

SEQ ID NO: 14 - protein, 518 aa, synthetic construct
GSHSMRYFYTAMSRPGRGEPRFIAVGYVDDTQFVRFDSDAASPRMEPRAPWIEQEGPEYWDGETRNMKASAQTYRENLRIALRYYNQSEAGSHIIQVMYGCDVGPDGRLLRGHDQSAYDGKDYIALNEDLSSWTAADTAAQITQRKWEAARVAEQLRAYLEGLCVEWLRRYLENGKETLQRADPPKTHVTHHPISDHEATLRCWALGFYPAEITLTWQRDGEDQTQDTELVETRPAGDRTFQKWAAVVVPSGEEQRYTCHVQHEGLPKPLTLRWEPSSQSGGGGSGGGGSESKYGPPCPPCPAPEFLGGPSVFLFPPKPKDTLMISRTPEVTCVVVDVSQEDPEVQFNWYVDGVEVHNAKTKPREEQFNSTYRVVSVLTVLHQDWLNGKEYKCKVSNKGLPSSIEKTISKAKGQPREPQVYTLPPSQEEMTKNQVSLTCLVKGFYPSDIAVEWESNGQPENNYKTTPPVLDSDGSFFLYSRLTVDKSRWQEGNVFSCSVMHEALHNHYTQKSLSLSLG

SEQ ID NO: 15 - protein, 518 aa, synthetic construct
GSHSMRYFYTAMSRPGRGEPRFIAVGYVDDTQFVRFDSDAASPRMAPRAPWIEQEGPEYWDGETRNMKASAQTYRENLRIALRYYNQSEAGSHIIQRMYGCDVGPDGRLLRGHDQSAYDGKDYIALNEDLSSWTAADTAAQITQRKWEAARVAEQLRAYLEGLCVEWLRRYLENGKETLQRADPPKTHVTHHPISDHEATLRCWALGFYPAEITLTWQRDGEDQTQDTELVETRPAGDRTFQKWAAVVVPSGEEQRYTCHVQHEGLPKPLTLRWEPSSQSGGGGSGGGGSESKYGPPCPPCPAPEFLGGPSVFLFPPKPKDTLMISRTPEVTCVVVDVSQEDPEVQFNWYVDGVEVHNAKTKPREEQFNSTYRVVSVLTVLHQDWLNGKEYKCKVSNKGLPSSIEKTISKAKGQPREPQVYTLPPSQEEMTKNQVSLTCLVKGFYPSDIAVEWESNGQPENNYKTTPPVLDSDGSFFLYSRLTVDKSRWQEGNVFSCSVMHEALHNHYTQKSLSLSLG

SEQ ID NO: 16 - protein, 518 aa, synthetic construct
GSHSMRYFYTAMSRPGRGEPRFIAVGYVDDTQFVRFDSDAASPRTAPRAPWIEQEGPEYWDGETRNMKASAQTYRENLRIALRYYNQSEAGSHIIQRMYGCDLGPDGRLLRGHDQSAYDGKDYIALNEDLSSWTAADTAAQITQRKWEAARVAEQLRAYLEGLCVEWLRRYLENGKETLQRADPPKTHVTHHPVSDHEATLRCWALGFYPAEITLTWQRDGEDQTQDTELVETRPAGDRTFQKWAAVVVPSGEEQRYTCHVQHEGLPKPLTLRWEPSSQSGGGGSGGGGSESKYGPPCPPCPAPEFLGGPSVFLFPPKPKDTLMISRTPEVTCVVVDVSQEDPEVQFNWYVDGVEVHNAKTKPREEQFNSTYRVVSVLTVLHQDWLNGKEYKCKVSNKGLPSSIEKTISKAKGQPREPQVYTLPPSQEEMTKNQVSLTCLVKGFYPSDIAVEWESNGQPENNYKTTPPVLDSDGSFFLYSRLTVDKSRWQEGNVFSCSVMHEALHNHYTQKSLSLSLG

SEQ ID NO: 17 - protein, 518 aa, synthetic construct
GSHSMRYFYTAMSRPGRGEPRFIAVGYVDDTQFVRFDSDAASPRTEPRAPWIEQEGPEYWDGETRNMKASAQTYRENLRIALRYYNQSEAGSHIIQVMYGCDLGPDGRLLRGHDQSAYDGKDYIALNEDLSSWTAADTAAQITQRKWEAARVAEQLRAYLEGLCVEWLRRYLENGKETLQRADPPKTHVTHHPVSDHEATLRCWALGFYPAEITLTWQRDGEDQTQDTELVETRPAGDRTFQKWAAVVVPSGEEQRYTCHVQHEGLPKPLTLRWEPSSQSGGGGSGGGGSESKYGPPCPPCPAPEFLGGPSVFLFPPKPKDTLMISRTPEVTCVVVDVSQEDPEVQFNWYVDGVEVHNAKTKPREEQFNSTYRVVSVLTVLHQDWLNGKEYKCKVSNKGLPSSIEKTISKAKGQPREPQVYTLPPSQEEMTKNQVSLTCLVKGFYPSDIAVEWESNGQPENNYKTTPPVLDSDGSFFLYSRLTVDKSRWQEGNVFSCSVMHEALHNHYTQKSLSLSLG

SEQ ID NO: 18 - protein, 518 aa, synthetic construct
GSHSMRYFYTAMSRPGRGEPRFIAVGYVDDTQFVRFDSDAASPRTAPRAPWIEQEGPEYWDGETRNMKASAQTYRENLRIALRYYNQSEAGSHIIQVMYGCDLGPDGRLLRGHDQSAYDGKDYIALNEDLSSWTAADTAAQITQRKWEAARVAEQLRAYLEGLCVEWLRRYLENGKETLQRADPPKTHVTHHPVSDHEATLRCWALGFYPAEITLTWQRDGEDQTQDTELVETRPAGDRTFQKWAAVVVPSGEEQRYTCHVQHEGLPKPLTLRWEPSSQSGGGGSGGGGSESKYGPPCPPCPAPEFLGGPSVFLFPPKPKDTLMISRTPEVTCVVVDVSQEDPEVQFNWYVDGVEVHNAKTKPREEQFNSTYRVVSVLTVLHQDWLNGKEYKCKVSNKGLPSSIEKTISKAKGQPREPQVYTLPPSQEEMTKNQVSLTCLVKGFYPSDIAVEWESNGQPENNYKTTPPVLDSDGSFFLYSRLTVDKSRWQEGNVFSCSVMHEALHNHYTQKSLSLSLG

SEQ ID NO: 19 - protein, 518 aa, synthetic construct
CSHSMRYFYTAVSRPGRGEPRFIAVGYVDDTQFVQFDSDAASPRGAPRAPWVEQEGPEYWDRETQKYKRQAQTDRVSLRNLRGYYNQSEAGSHTLQRMYGCDLGPDGRLLRGYNQFAYDGKDYIALNEDLRSWTAADKAAQITQRKWEAAREAEQRRAYLEGTCVEWLRRYLENGKKTLQRAEHPKTHVTHHPVSDHEATLRCWALGFYPAEITLTWQRDGEDQTQDTELVETRPAGDGTFQKWAAVVVPSGEEQRYTCHVQHEGLPEPLTLRWGPSSQPGGGGSGGGGSESKYGPPCPPCPAPEFLGGPSVFLFPPKPKDTLMISRTPEVTCVVVDVSQEDPEVQFNWYVDGVEVHNAKTKPREEQFNSTYRVVSVLTVLHQDWLNGKEYKCKVSNKGLPSSIEKTISKAKGQPREPQVYTLPPSQEEMTKNQVSLTCLVKGFYPSDIAVEWESNGQPENNYKTTPPVLDSDGSFFLYSRLTVDKSRWQEGNVFSCSVMHEALHNHYTQKSLSLSLG

SEQ ID NO: 20 - protein, 518 aa, synthetic construct
CSHSMRYFYTAVSRPGRGEPRFIAVGYVDDTQFVQFDSDAASPRGEPRAPWVEQEGPEYWDRETQKYKRQAQTDRVSLRNLRGYYNQSEAGSHTLQVMYGCDLGPDGRLLRGYNQFAYDGKDYIALNEDLRSWTAADKAAQITQRKWEAAREAEQRRAYLEGTCVEWLRRYLENGKKTLQRAEHPKTHVTHHPVSDHEATLRCWALGFYPAEITLTWQRDGEDQTQDTELVETRPAGDGTFQKWAAVVVPSGEEQRYTCHVQHEGLPEPLTLRWGPSSQPGGGGSGGGGSESKYGPPCPPCPAPEFLGGPSVFLFPPKPKDTLMISRTPEVTCVVVDVSQEDPEVQFNWYVDGVEVHNAKTKPREEQFNSTYRVVSVLTVLHQDWLNGKEYKCKVSNKGLPSSIEKTISKAKGQPREPQVYTLPPSQEEMTKNQVSLTCLVKGFYPSDIAVEWESNGQPENNYKTTPPVLDSDGSFFLYSRLTVDKSRWQEGNVFSCSVMHEALHNHYTQKSLSLSLG

SEQ ID NO: 21 - protein, 518 aa, synthetic construct
CSHSMRYFYTAVSRPGRGEPRFIAVGYVDDTQFVQFDSDAASPRGAPRAPWVEQEGPEYWDRETQKYKRQAQTDRVSLRNLRGYYNQSEAGSHTLQVMYGCDLGPDGRLLRGYNQFAYDGKDYIALNEDLRSWTAADKAAQITQRKWEAAREAEQRRAYLEGTCVEWLRRYLENGKKTLQRAEHPKTHVTHHPVSDHEATLRCWALGFYPAEITLTWQRDGEDQTQDTELVETRPAGDGTFQKWAAVVVPSGEEQRYTCHVQHEGLPEPLTLRWGPSSQPGGGGSGGGGSESKYGPPCPPCPAPEFLGGPSVFLFPPKPKDTLMISRTPEVTCVVVDVSQEDPEVQFNWYVDGVEVHNAKTKPREEQFNSTYRVVSVLTVLHQDWLNGKEYKCKVSNKGLPSSIEKTISKAKGQPREPQVYTLPPSQEEMTKNQVSLTCLVKGFYPSDIAVEWESNGQPENNYKTTPPVLDSDGSFFLYSRLTVDKSRWQEGNVFSCSVMHEALHNHYTQKSLSLSLG